European Patent Application EP 4 461 821 A2, published November 13, 2024. Title: POLYMERASE COMPOSITIONS AND METHODS OF MAKING AND USING SAME. Applicant: LIFE TECHNOLOGIES CORPORATION. Application EP. The sequence listing filed with the application follows.

SEQUENCE LISTING (44 sequences)

SEQ ID NO: 1 - protein, 832 aa, Thermus aquaticus [sequence omitted]

SEQ ID NO: 2 - protein, 832 aa, synthetic construct
  REGION 1..832: note = Synthetic: Taq mutant E397V (Hit #1)
MRGMLPLFEPKGRVLLVDGHHLAYRTFHALKGLTTSRGEPVQAVYGFAKSLLKALKEDGDAVIVVFDAKAPSFRHEAYGGYKAGRAPTPEDFPRQLALIKELVDLLGLARLEVPGYEADDVLASLAKKAEKEGYEVRILTADKDLYQLLSDRIHVLHPEGYLITPAWLWEKYGLRPDQWADYRALTGDESDNLPGVKGIGEKTARKLLEEWGSLEALLKNLDRLKPAIREKILAHMDDLKLSWDLAKVRTDLPLEVDFAKRREPDRERLRAFLERLEFGSLLHEFGLLESPKALEEAPWPPPEGAFVGFVLSRKEPMWADLLALAAARGGRVHRAPEPYKALRDLKEARGLLAKDLSVLALREGLGLPPGDDPMLLAYLLDPSNTTPEGVARRYGGVWTEEAGERAALSERLFANLWGRLEGEERLLWLYREVERPLSAVLAHMEATGVRLDVAYLRALSLEVAEEIARLEAEVFRLAGHPFNLNSRDQLERVLFDELGLPAIGKTEKTGKRSTSAAVLEALREAHPIVEKILQYRELTKLKSTYIDPLPDLIHPRTGRLHTRFNQTATATGRLSSSDPNLQNIPVRTPLGQRIRRAFIAEEGWLLVALDYSQIELRVLAHLSGDENLIRVFQEGRDIHTETASWMFGVPREAVDPLMRRAAKTINFGVLYGMSAHRLSQELAIPYEEAQAFIERYFQSFPKVRAWIEKTLEEGRRRGYVETLFGRRRYVPDLEARVKSVREAAERMAFNMPVQGTAADLMKLAMVKLFPRLEEMGARMLLQVHDELVLEAPKERAEAVARLAKEVMEGVYPLAVPLEVEVGIGEDWLSAKE

SEQ ID NO: 3 - protein, 832 aa, synthetic construct
  REGION 1..832: note = Synthetic: (L763F + E805I)
MRGMLPLFEPKGRVLLVDGHHLAYRTFHALKGLTTSRGEPVQAVYGFAKSLLKALKEDGDAVIVVFDAKAPSFRHEAYGGYKAGRAPTPEDFPRQLALIKELVDLLGLARLEVPGYEADDVLASLAKKAEKEGYEVRILTADKDLYQLLSDRIHVLHPEGYLITPAWLWEKYGLRPDQWADYRALTGDESDNLPGVKGIGEKTARKLLEEWGSLEALLKNLDRLKPAIREKILAHMDDLKLSWDLAKVRTDLPLEVDFAKRREPDRERLRAFLERLEFGSLLHEFGLLESPKALEEAPWPPPEGAFVGFVLSRKEPMWADLLALAAARGGRVHRAPEPYKALRDLKEARGLLAKDLSVLALREGLGLPPGDDPMLLAYLLDPSNTTPEGVARRYGGEWTEEAGERAALSERLFANLWGRLEGEERLLWLYREVERPLSAVLAHMEATGVRLDVAYLRALSLEVAEEIARLEAEVFRLAGHPFNLNSRDQLERVLFDELGLPAIGKTEKTGKRSTSAAVLEALREAHPIVEKILQYRELTKLKSTYIDPLPDLIHPRTGRLHTRFNQTATATGRLSSSDPNLQNIPVRTPLGQRIRRAFIAEEGWLLVALDYSQIELRVLAHLSGDENLIRVFQEGRDIHTETASWMFGVPREAVDPLMRRAAKTINFGVLYGMSAHRLSQELAIPYEEAQAFIERYFQSFPKVRAWIEKTLEEGRRRGYVETLFGRRRYVPDLEARVKSVREAAERMAFNMPVQGTAADLMKFAMVKLFPRLEEMGARMLLQVHDELVLEAPKERAEAVARLAKIVMEGVYPLAVPLEVEVGIGEDWLSAKE

SEQ ID NO: 4 - protein, 832 aa, synthetic construct
  REGION 1..832: note = Synthetic: (E397V + E745T + L763F)
MRGMLPLFEPKGRVLLVDGHHLAYRTFHALKGLTTSRGEPVQAVYGFAKSLLKALKEDGDAVIVVFDAKAPSFRHEAYGGYKAGRAPTPEDFPRQLALIKELVDLLGLARLEVPGYEADDVLASLAKKAEKEGYEVRILTADKDLYQLLSDRIHVLHPEGYLITPAWLWEKYGLRPDQWADYRALTGDESDNLPGVKGIGEKTARKLLEEWGSLEALLKNLDRLKPAIREKILAHMDDLKLSWDLAKVRTDLPLEVDFAKRREPDRERLRAFLERLEFGSLLHEFGLLESPKALEEAPWPPPEGAFVGFVLSRKEPMWADLLALAAARGGRVHRAPEPYKALRDLKEARGLLAKDLSVLALREGLGLPPGDDPMLLAYLLDPSNTTPEGVARRYGGVWTEEAGERAALSERLFANLWGRLEGEERLLWLYREVERPLSAVLAHMEATGVRLDVAYLRALSLEVAEEIARLEAEVFRLAGHPFNLNSRDQLERVLFDELGLPAIGKTEKTGKRSTSAAVLEALREAHPIVEKILQYRELTKLKSTYIDPLPDLIHPRTGRLHTRFNQTATATGRLSSSDPNLQNIPVRTPLGQRIRRAFIAEEGWLLVALDYSQIELRVLAHLSGDENLIRVFQEGRDIHTETASWMFGVPREAVDPLMRRAAKTINFGVLYGMSAHRLSQELAIPYEEAQAFIERYFQSFPKVRAWIEKTLEEGRRRGYVETLFGRRRYVPDLEARVKSVREAATRMAFNMPVQGTAADLMKFAMVKLFPRLEEMGARMLLQVHDELVLEAPKERAEAVARLAKEVMEGVYPLAVPLEVEVGIGEDWLSAKE

SEQ ID NO: 5 - protein, 832 aa, synthetic construct
  REGION 1..832: note = Synthetic: P6N
MRGMLNLFEPKGRVLLVDGHHLAYRTFHALKGLTTSRGEPVQAVYGFAKSLLKALKEDGDAVIVVFDAKAPSFRHEAYGGYKAGRAPTPEDFPRQLALIKELVDLLGLARLEVPGYEADDVLASLAKKAEKEGYEVRILTADKDLYQLLSDRIHVLHPEGYLITPAWLWEKYGLRPDQWADYRALTGDESDNLPGVKGIGEKTARKLLEEWGSLEALLKNLDRLKPAIREKILAHMDDLKLSWDLAKVRTDLPLEVDFAKRREPDRERLRAFLERLEFGSLLHEFGLLESPKALEEAPWPPPEGAFVGFVLSRKEPMWADLLALAAARGGRVHRAPEPYKALRDLKEARGLLAKDLSVLALREGLGLPPGDDPMLLAYLLDPSNTTPEGVARRYGGEWTEEAGERAALSERLFANLWGRLEGEERLLWLYREVERPLSAVLAHMEATGVRLDVAYLRALSLEVAEEIARLEAEVFRLAGHPFNLNSRDQLERVLFDELGLPAIGKTEKTGKRSTSAAVLEALREAHPIVEKILQYRELTKLKSTYIDPLPDLIHPRTGRLHTRFNQTATATGRLSSSDPNLQNIPVRTPLGQRIRRAFIAEEGWLLVALDYSQIELRVLAHLSGDENLIRVFQEGRDIHTETASWMFGVPREAVDPLMRRAAKTINFGVLYGMSAHRLSQELAIPYEEAQAFIERYFQSFPKVRAWIEKTLEEGRRRGYVETLFGRRRYVPDLEARVKSVREAAERMAFNMPVQGTAADLMKLAMVKLFPRLEEMGARMLLQVHDELVLEAPKERAEAVARLAKEVMEGVYPLAVPLEVEVGIGEDWLSAKE

SEQ ID NO: 6 - protein, 832 aa, synthetic construct
  REGION 1..832: note = Synthetic: A77E
MRGMLPLFEPKGRVLLVDGHHLAYRTFHALKGLTTSRGEPVQAVYGFAKSLLKALKEDGDAVIVVFDAKAPSFRHEEYGGYKAGRAPTPEDFPRQLALIKELVDLLGLARLEVPGYEADDVLASLAKKAEKEGYEVRILTADKDLYQLLSDRIHVLHPEGYLITPAWLWEKYGLRPDQWADYRALTGDESDNLPGVKGIGEKTARKLLEEWGSLEALLKNLDRLKPAIREKILAHMDDLKLSWDLAKVRTDLPLEVDFAKRREPDRERLRAFLERLEFGSLLHEFGLLESPKALEEAPWPPPEGAFVGFVLSRKEPMWADLLALAAARGGRVHRAPEPYKALRDLKEARGLLAKDLSVLALREGLGLPPGDDPMLLAYLLDPSNTTPEGVARRYGGEWTEEAGERAALSERLFANLWGRLEGEERLLWLYREVERPLSAVLAHMEATGVRLDVAYLRALSLEVAEEIARLEAEVFRLAGHPFNLNSRDQLERVLFDELGLPAIGKTEKTGKRSTSAAVLEALREAHPIVEKILQYRELTKLKSTYIDPLPDLIHPRTGRLHTRFNQTATATGRLSSSDPNLQNIPVRTPLGQRIRRAFIAEEGWLLVALDYSQIELRVLAHLSGDENLIRVFQEGRDIHTETASWMFGVPREAVDPLMRRAAKTINFGVLYGMSAHRLSQELAIPYEEAQAFIERYFQSFPKVRAWIEKTLEEGRRRGYVETLFGRRRYVPDLEARVKSVREAAERMAFNMPVQGTAADLMKLAMVKLFPRLEEMGARMLLQVHDELVLEAPKERAEAVARLAKEVMEGVYPLAVPLEVEVGIGEDWLSAKE

SEQ ID NO: 7 - protein, 832 aa, synthetic construct
  REGION 1..832: note = Synthetic: A97V
MRGMLPLFEPKGRVLLVDGHHLAYRTFHALKGLTTSRGEPVQAVYGFAKSLLKALKEDGDAVIVVFDAKAPSFRHEAYGGYKAGRAPTPEDFPRQLVLIKELVDLLGLARLEVPGYEADDVLASLAKKAEKEGYEVRILTADKDLYQLLSDRIHVLHPEGYLITPAWLWEKYGLRPDQWADYRALTGDESDNLPGVKGIGEKTARKLLEEWGSLEALLKNLDRLKPAIREKILAHMDDLKLSWDLAKVRTDLPLEVDFAKRREPDRERLRAFLERLEFGSLLHEFGLLESPKALEEAPWPPPEGAFVGFVLSRKEPMWADLLALAAARGGRVHRAPEPYKALRDLKEARGLLAKDLSVLALREGLGLPPGDDPMLLAYLLDPSNTTPEGVARRYGGEWTEEAGERAALSERLFANLWGRLEGEERLLWLYREVERPLSAVLAHMEATGVRLDVAYLRALSLEVAEEIARLEAEVFRLAGHPFNLNSRDQLERVLFDELGLPAIGKTEKTGKRSTSAAVLEALREAHPIVEKILQYRELTKLKSTYIDPLPDLIHPRTGRLHTRFNQTATATGRLSSSDPNLQNIPVRTPLGQRIRRAFIAEEGWLLVALDYSQIELRVLAHLSGDENLIRVFQEGRDIHTETASWMFGVPREAVDPLMRRAAKTINFGVLYGMSAHRLSQELAIPYEEAQAFIERYFQSFPKVRAWIEKTLEEGRRRGYVETLFGRRRYVPDLEARVKSVREAAERMAFNMPVQGTAADLMKLAMVKLFPRLEEMGARMLLQVHDELVLEAPKERAEAVARLAKEVMEGVYPLAVPLEVEVGIGEDWLSAKE

SEQ ID NO: 8 - protein, 832 aa, synthetic construct
  REGION 1..832: note = Synthetic: L193V
MRGMLPLFEPKGRVLLVDGHHLAYRTFHALKGLTTSRGEPVQAVYGFAKSLLKALKEDGDAVIVVFDAKAPSFRHEAYGGYKAGRAPTPEDFPRQLALIKELVDLLGLARLEVPGYEADDVLASLAKKAEKEGYEVRILTADKDLYQLLSDRIHVLHPEGYLITPAWLWEKYGLRPDQWADYRALTGDESDNVPGVKGIGEKTARKLLEEWGSLEALLKNLDRLKPAIREKILAHMDDLKLSWDLAKVRTDLPLEVDFAKRREPDRERLRAFLERLEFGSLLHEFGLLESPKALEEAPWPPPEGAFVGFVLSRKEPMWADLLALAAARGGRVHRAPEPYKALRDLKEARGLLAKDLSVLALREGLGLPPGDDPMLLAYLLDPSNTTPEGVARRYGGEWTEEAGERAALSERLFANLWGRLEGEERLLWLYREVERPLSAVLAHMEATGVRLDVAYLRALSLEVAEEIARLEAEVFRLAGHPFNLNSRDQLERVLFDELGLPAIGKTEKTGKRSTSAAVLEALREAHPIVEKILQYRELTKLKSTYIDPLPDLIHPRTGRLHTRFNQTATATGRLSSSDPNLQNIPVRTPLGQRIRRAFIAEEGWLLVALDYSQIELRVLAHLSGDENLIRVFQEGRDIHTETASWMFGVPREAVDPLMRRAAKTINFGVLYGMSAHRLSQELAIPYEEAQAFIERYFQSFPKVRAWIEKTLEEGRRRGYVETLFGRRRYVPDLEARVKSVREAAERMAFNMPVQGTAADLMKLAMVKLFPRLEEMGARMLLQVHDELVLEAPKERAEAVARLAKEVMEGVYPLAVPLEVEVGIGEDWLSAKE

SEQ ID NO: 9 - protein, 832 aa, synthetic construct
  REGION 1..832: note = Synthetic: K240I
MRGMLPLFEPKGRVLLVDGHHLAYRTFHALKGLTTSRGEPVQAVYGFAKSLLKALKEDGDAVIVVFDAKAPSFRHEAYGGYKAGRAPTPEDFPRQLALIKELVDLLGLARLEVPGYEADDVLASLAKKAEKEGYEVRILTADKDLYQLLSDRIHVLHPEGYLITPAWLWEKYGLRPDQWADYRALTGDESDNLPGVKGIGEKTARKLLEEWGSLEALLKNLDRLKPAIREKILAHMDDLILSWDLAKVRTDLPLEVDFAKRREPDRERLRAFLERLEFGSLLHEFGLLESPKALEEAPWPPPEGAFVGFVLSRKEPMWADLLALAAARGGRVHRAPEPYKALRDLKEARGLLAKDLSVLALREGLGLPPGDDPMLLAYLLDPSNTTPEGVARRYGGEWTEEAGERAALSERLFANLWGRLEGEERLLWLYREVERPLSAVLAHMEATGVRLDVAYLRALSLEVAEEIARLEAEVFRLAGHPFNLNSRDQLERVLFDELGLPAIGKTEKTGKRSTSAAVLEALREAHPIVEKILQYRELTKLKSTYIDPLPDLIHPRTGRLHTRFNQTATATGRLSSSDPNLQNIPVRTPLGQRIRRAFIAEEGWLLVALDYSQIELRVLAHLSGDENLIRVFQEGRDIHTETASWMFGVPREAVDPLMRRAAKTINFGVLYGMSAHRLSQELAIPYEEAQAFIERYFQSFPKVRAWIEKTLEEGRRRGYVETLFGRRRYVPDLEARVKSVREAAERMAFNMPVQGTAADLMKLAMVKLFPRLEEMGARMLLQVHDELVLEAPKERAEAVARLAKEVMEGVYPLAVPLEVEVGIGEDWLSAKE

SEQ ID NO: 10 - protein, 832 aa, synthetic construct
  REGION 1..832: note = Synthetic: R266Q
MRGMLPLFEPKGRVLLVDGHHLAYRTFHALKGLTTSRGEPVQAVYGFAKSLLKALKEDGDAVIVVFDAKAPSFRHEAYGGYKAGRAPTPEDFPRQLALIKELVDLLGLARLEVPGYEADDVLASLAKKAEKEGYEVRILTADKDLYQLLSDRIHVLHPEGYLITPAWLWEKYGLRPDQWADYRALTGDESDNLPGVKGIGEKTARKLLEEWGSLEALLKNLDRLKPAIREKILAHMDDLKLSWDLAKVRTDLPLEVDFAKRREPDQERLRAFLERLEFGSLLHEFGLLESPKALEEAPWPPPEGAFVGFVLSRKEPMWADLLALAAARGGRVHRAPEPYKALRDLKEARGLLAKDLSVLALREGLGLPPGDDPMLLAYLLDPSNTTPEGVARRYGGEWTEEAGERAALSERLFANLWGRLEGEERLLWLYREVERPLSAVLAHMEATGVRLDVAYLRALSLEVAEEIARLEAEVFRLAGHPFNLNSRDQLERVLFDELGLPAIGKTEKTGKRSTSAAVLEALREAHPIVEKILQYRELTKLKSTYIDPLPDLIHPRTGRLHTRFNQTATATGRLSSSDPNLQNIPVRTPLGQRIRRAFIAEEGWLLVALDYSQIELRVLAHLSGDENLIRVFQEGRDIHTETASWMFGVPREAVDPLMRRAAKTINFGVLYGMSAHRLSQELAIPYEEAQAFIERYFQSFPKVRAWIEKTLEEGRRRGYVETLFGRRRYVPDLEARVKSVREAAERMAFNMPVQGTAADLMKLAMVKLFPRLEEMGARMLLQVHDELVLEAPKERAEAVARLAKEVMEGVYPLAVPLEVEVGIGEDWLSAKE

SEQ ID NO: 11 - protein, 832 aa, synthetic construct
  REGION 1..832: note = Synthetic: E267T
MRGMLPLFEPKGRVLLVDGHHLAYRTFHALKGLTTSRGEPVQAVYGFAKSLLKALKEDGDAVIVVFDAKAPSFRHEAYGGYKAGRAPTPEDFPRQLALIKELVDLLGLARLEVPGYEADDVLASLAKKAEKEGYEVRILTADKDLYQLLSDRIHVLHPEGYLITPAWLWEKYGLRPDQWADYRALTGDESDNLPGVKGIGEKTARKLLEEWGSLEALLKNLDRLKPAIREKILAHMDDLKLSWDLAKVRTDLPLEVDFAKRREPDRTRLRAFLERLEFGSLLHEFGLLESPKALEEAPWPPPEGAFVGFVLSRKEPMWADLLALAAARGGRVHRAPEPYKALRDLKEARGLLAKDLSVLALREGLGLPPGDDPMLLAYLLDPSNTTPEGVARRYGGEWTEEAGERAALSERLFANLWGRLEGEERLLWLYREVERPLSAVLAHMEATGVRLDVAYLRALSLEVAEEIARLEAEVFRLAGHPFNLNSRDQLERVLFDELGLPAIGKTEKTGKRSTSAAVLEALREAHPIVEKILQYRELTKLKSTYIDPLPDLIHPRTGRLHTRFNQTATATGRLSSSDPNLQNIPVRTPLGQRIRRAFIAEEGWLLVALDYSQIELRVLAHLSGDENLIRVFQEGRDIHTETASWMFGVPREAVDPLMRRAAKTINFGVLYGMSAHRLSQELAIPYEEAQAFIERYFQSFPKVRAWIEKTLEEGRRRGYVETLFGRRRYVPDLEARVKSVREAAERMAFNMPVQGTAADLMKLAMVKLFPRLEEMGARMLLQVHDELVLEAPKERAEAVARLAKEVMEGVYPLAVPLEVEVGIGEDWLSAKE

SEQ ID NO: 12 - protein, 832 aa, synthetic construct
  REGION 1..832: note = Synthetic: L287T
MRGMLPLFEPKGRVLLVDGHHLAYRTFHALKGLTTSRGEPVQAVYGFAKSLLKALKEDGDAVIVVFDAKAPSFRHEAYGGYKAGRAPTPEDFPRQLALIKELVDLLGLARLEVPGYEADDVLASLAKKAEKEGYEVRILTADKDLYQLLSDRIHVLHPEGYLITPAWLWEKYGLRPDQWADYRALTGDESDNLPGVKGIGEKTARKLLEEWGSLEALLKNLDRLKPAIREKILAHMDDLKLSWDLAKVRTDLPLEVDFAKRREPDRERLRAFLERLEFGSLLHEFGTLESPKALEEAPWPPPEGAFVGFVLSRKEPMWADLLALAAARGGRVHRAPEPYKALRDLKEARGLLAKDLSVLALREGLGLPPGDDPMLLAYLLDPSNTTPEGVARRYGGEWTEEAGERAALSERLFANLWGRLEGEERLLWLYREVERPLSAVLAHMEATGVRLDVAYLRALSLEVAEEIARLEAEVFRLAGHPFNLNSRDQLERVLFDELGLPAIGKTEKTGKRSTSAAVLEALREAHPIVEKILQYRELTKLKSTYIDPLPDLIHPRTGRLHTRFNQTATATGRLSSSDPNLQNIPVRTPLGQRIRRAFIAEEGWLLVALDYSQIELRVLAHLSGDENLIRVFQEGRDIHTETASWMFGVPREAVDPLMRRAAKTINFGVLYGMSAHRLSQELAIPYEEAQAFIERYFQSFPKVRAWIEKTLEEGRRRGYVETLFGRRRYVPDLEARVKSVREAAERMAFNMPVQGTAADLMKLAMVKLFPRLEEMGARMLLQVHDELVLEAPKERAEAVARLAKEVMEGVYPLAVPLEVEVGIGEDWLSAKE

SEQ ID NO: 13 - protein, 832 aa, synthetic construct
  REGION 1..832: note = Synthetic: P291T
MRGMLPLFEPKGRVLLVDGHHLAYRTFHALKGLTTSRGEPVQAVYGFAKSLLKALKEDGDAVIVVFDAKAPSFRHEAYGGYKAGRAPTPEDFPRQLALIKELVDLLGLARLEVPGYEADDVLASLAKKAEKEGYEVRILTADKDLYQLLSDRIHVLHPEGYLITPAWLWEKYGLRPDQWADYRALTGDESDNLPGVKGIGEKTARKLLEEWGSLEALLKNLDRLKPAIREKILAHMDDLKLSWDLAKVRTDLPLEVDFAKRREPDRERLRAFLERLEFGSLLHEFGLLESTKALEEAPWPPPEGAFVGFVLSRKEPMWADLLALAAARGGRVHRAPEPYKALRDLKEARGLLAKDLSVLALREGLGLPPGDDPMLLAYLLDPSNTTPEGVARRYGGEWTEEAGERAALSERLFANLWGRLEGEERLLWLYREVERPLSAVLAHMEATGVRLDVAYLRALSLEVAEEIARLEAEVFRLAGHPFNLNSRDQLERVLFDELGLPAIGKTEKTGKRSTSAAVLEALREAHPIVEKILQYRELTKLKSTYIDPLPDLIHPRTGRLHTRFNQTATATGRLSSSDPNLQNIPVRTPLGQRIRRAFIAEEGWLLVALDYSQIELRVLAHLSGDENLIRVFQEGRDIHTETASWMFGVPREAVDPLMRRAAKTINFGVLYGMSAHRLSQELAIPYEEAQAFIERYFQSFPKVRAWIEKTLEEGRRRGYVETLFGRRRYVPDLEARVKSVREAAERMAFNMPVQGTAADLMKLAMVKLFPRLEEMGARMLLQVHDELVLEAPKERAEAVARLAKEVMEGVYPLAVPLEVEVGIGEDWLSAKE

SEQ ID NO: 14 - protein, 832 aa, synthetic construct
  REGION 1..832: note = Synthetic: K292C
MRGMLPLFEPKGRVLLVDGHHLAYRTFHALKGLTTSRGEPVQAVYGFAKSLLKALKEDGDAVIVVFDAKAPSFRHEAYGGYKAGRAPTPEDFPRQLALIKELVDLLGLARLEVPGYEADDVLASLAKKAEKEGYEVRILTADKDLYQLLSDRIHVLHPEGYLITPAWLWEKYGLRPDQWADYRALTGDESDNLPGVKGIGEKTARKLLEEWGSLEALLKNLDRLKPAIREKILAHMDDLKLSWDLAKVRTDLPLEVDFAKRREPDRERLRAFLERLEFGSLLHEFGLLESPCALEEAPWPPPEGAFVGFVLSRKEPMWADLLALAAARGGRVHRAPEPYKALRDLKEARGLLAKDLSVLALREGLGLPPGDDPMLLAYLLDPSNTTPEGVARRYGGEWTEEAGERAALSERLFANLWGRLEGEERLLWLYREVERPLSAVLAHMEATGVRLDVAYLRALSLEVAEEIARLEAEVFRLAGHPFNLNSRDQLERVLFDELGLPAIGKTEKTGKRSTSAAVLEALREAHPIVEKILQYRELTKLKSTYIDPLPDLIHPRTGRLHTRFNQTATATGRLSSSDPNLQNIPVRTPLGQRIRRAFIAEEGWLLVALDYSQIELRVLAHLSGDENLIRVFQEGRDIHTETASWMFGVPREAVDPLMRRAAKTINFGVLYGMSAHRLSQELAIPYEEAQAFIERYFQSFPKVRAWIEKTLEEGRRRGYVETLFGRRRYVPDLEARVKSVREAAERMAFNMPVQGTAADLMKLAMVKLFPRLEEMGARMLLQVHDELVLEAPKERAEAVARLAKEVMEGVYPLAVPLEVEVGIGEDWLSAKE

SEQ ID NO: 15 - protein, 832 aa, synthetic construct
  REGION 1..832: note = Synthetic: E295F
MRGMLPLFEPKGRVLLVDGHHLAYRTFHALKGLTTSRGEPVQAVYGFAKSLLKALKEDGDAVIVVFDAKAPSFRHEAYGGYKAGRAPTPEDFPRQLALIKELVDLLGLARLEVPGYEADDVLASLAKKAEKEGYEVRILTADKDLYQLLSDRIHVLHPEGYLITPAWLWEKYGLRPDQWADYRALTGDESDNLPGVKGIGEKTARKLLEEWGSLEALLKNLDRLKPAIREKILAHMDDLKLSWDLAKVRTDLPLEVDFAKRREPDRERLRAFLERLEFGSLLHEFGLLESPKALFEAPWPPPEGAFVGFVLSRKEPMWADLLALAAARGGRVHRAPEPYKALRDLKEARGLLAKDLSVLALREGLGLPPGDDPMLLAYLLDPSNTTPEGVARRYGGEWTEEAGERAALSERLFANLWGRLEGEERLLWLYREVERPLSAVLAHMEATGVRLDVAYLRALSLEVAEEIARLEAEVFRLAGHPFNLNSRDQLERVLFDELGLPAIGKTEKTGKRSTSAAVLEALREAHPIVEKILQYRELTKLKSTYIDPLPDLIHPRTGRLHTRFNQTATATGRLSSSDPNLQNIPVRTPLGQRIRRAFIAEEGWLLVALDYSQIELRVLAHLSGDENLIRVFQEGRDIHTETASWMFGVPREAVDPLMRRAAKTINFGVLYGMSAHRLSQELAIPYEEAQAFIERYFQSFPKVRAWIEKTLEEGRRRGYVETLFGRRRYVPDLEARVKSVREAAERMAFNMPVQGTAADLMKLAMVKLFPRLEEMGARMLLQVHDELVLEAPKERAEAVARLAKEVMEGVYPLAVPLEVEVGIGEDWLSAKE

SEQ ID NO: 16 - protein, 832 aa, synthetic construct
  REGION 1..832: note = Synthetic: E295N
MRGMLPLFEPKGRVLLVDGHHLAYRTFHALKGLTTSRGEPVQAVYGFAKSLLKALKEDGDAVIVVFDAKAPSFRHEAYGGYKAGRAPTPEDFPRQLALIKELVDLLGLARLEVPGYEADDVLASLAKKAEKEGYEVRILTADKDLYQLLSDRIHVLHPEGYLITPAWLWEKYGLRPDQWADYRALTGDESDNLPGVKGIGEKTARKLLEEWGSLEALLKNLDRLKPAIREKILAHMDDLKLSWDLAKVRTDLPLEVDFAKRREPDRERLRAFLERLEFGSLLHEFGLLESPKALNEAPWPPPEGAFVGFVLSRKEPMWADLLALAAARGGRVHRAPEPYKALRDLKEARGLLAKDLSVLALREGLGLPPGDDPMLLAYLLDPSNTTPEGVARRYGGEWTEEAGERAALSERLFANLWGRLEGEERLLWLYREVERPLSAVLAHMEATGVRLDVAYLRALSLEVAEEIARLEAEVFRLAGHPFNLNSRDQLERVLFDELGLPAIGKTEKTGKRSTSAAVLEALREAHPIVEKILQYRELTKLKSTYIDPLPDLIHPRTGRLHTRFNQTATATGRLSSSDPNLQNIPVRTPLGQRIRRAFIAEEGWLLVALDYSQIELRVLAHLSGDENLIRVFQEGRDIHTETASWMFGVPREAVDPLMRRAAKTINFGVLYGMSAHRLSQELAIPYEEAQAFIERYFQSFPKVRAWIEKTLEEGRRRGYVETLFGRRRYVPDLEARVKSVREAAERMAFNMPVQGTAADLMKLAMVKLFPRLEEMGARMLLQVHDELVLEAPKERAEAVARLAKEVMEGVYPLAVPLEVEVGIGEDWLSAKE

SEQ ID NO: 17 - protein, 832 aa, synthetic construct
  REGION 1..832: note = Synthetic: G418C
MRGMLPLFEPKGRVLLVDGHHLAYRTFHALKGLTTSRGEPVQAVYGFAKSLLKALKEDGDAVIVVFDAKAPSFRHEAYGGYKAGRAPTPEDFPRQLALIKELVDLLGLARLEVPGYEADDVLASLAKKAEKEGYEVRILTADKDLYQLLSDRIHVLHPEGYLITPAWLWEKYGLRPDQWADYRALTGDESDNLPGVKGIGEKTARKLLEEWGSLEALLKNLDRLKPAIREKILAHMDDLKLSWDLAKVRTDLPLEVDFAKRREPDRERLRAFLERLEFGSLLHEFGLLESPKALEEAPWPPPEGAFVGFVLSRKEPMWADLLALAAARGGRVHRAPEPYKALRDLKEARGLLAKDLSVLALREGLGLPPGDDPMLLAYLLDPSNTTPEGVARRYGGEWTEEAGERAALSERLFANLWCRLEGEERLLWLYREVERPLSAVLAHMEATGVRLDVAYLRALSLEVAEEIARLEAEVFRLAGHPFNLNSRDQLERVLFDELGLPAIGKTEKTGKRSTSAAVLEALREAHPIVEKILQYRELTKLKSTYIDPLPDLIHPRTGRLHTRFNQTATATGRLSSSDPNLQNIPVRTPLGQRIRRAFIAEEGWLLVALDYSQIELRVLAHLSGDENLIRVFQEGRDIHTETASWMFGVPREAVDPLMRRAAKTINFGVLYGMSAHRLSQELAIPYEEAQAFIERYFQSFPKVRAWIEKTLEEGRRRGYVETLFGRRRYVPDLEARVKSVREAAERMAFNMPVQGTAADLMKLAMVKLFPRLEEMGARMLLQVHDELVLEAPKERAEAVARLAKEVMEGVYPLAVPLEVEVGIGEDWLSAKE

SEQ ID NO: 18 - protein, 832 aa, synthetic construct
  REGION 1..832: note = Synthetic: L490Q
MRGMLPLFEPKGRVLLVDGHHLAYRTFHALKGLTTSRGEPVQAVYGFAKSLLKALKEDGDAVIVVFDAKAPSFRHEAYGGYKAGRAPTPEDFPRQLALIKELVDLLGLARLEVPGYEADDVLASLAKKAEKEGYEVRILTADKDLYQLLSDRIHVLHPEGYLITPAWLWEKYGLRPDQWADYRALTGDESDNLPGVKGIGEKTARKLLEEWGSLEALLKNLDRLKPAIREKILAHMDDLKLSWDLAKVRTDLPLEVDFAKRREPDRERLRAFLERLEFGSLLHEFGLLESPKALEEAPWPPPEGAFVGFVLSRKEPMWADLLALAAARGGRVHRAPEPYKALRDLKEARGLLAKDLSVLALREGLGLPPGDDPMLLAYLLDPSNTTPEGVARRYGGEWTEEAGERAALSERLFANLWGRLEGEERLLWLYREVERPLSAVLAHMEATGVRLDVAYLRALSLEVAEEIARLEAEVFRLAGHPFNLNSRDQQERVLFDELGLPAIGKTEKTGKRSTSAAVLEALREAHPIVEKILQYRELTKLKSTYIDPLPDLIHPRTGRLHTRFNQTATATGRLSSSDPNLQNIPVRTPLGQRIRRAFIAEEGWLLVALDYSQIELRVLAHLSGDENLIRVFQEGRDIHTETASWMFGVPREAVDPLMRRAAKTINFGVLYGMSAHRLSQELAIPYEEAQAFIERYFQSFPKVRAWIEKTLEEGRRRGYVETLFGRRRYVPDLEARVKSVREAAERMAFNMPVQGTAADLMKLAMVKLFPRLEEMGARMLLQVHDELVLEAPKERAEAVARLAKEVMEGVYPLAVPLEVEVGIGEDWLSAKE

SEQ ID NO: 19 - protein, 832 aa, synthetic construct
  REGION 1..832: note = Synthetic: A502S
MRGMLPLFEPKGRVLLVDGHHLAYRTFHALKGLTTSRGEPVQAVYGFAKSLLKALKEDGDAVIVVFDAKAPSFRHEAYGGYKAGRAPTPEDFPRQLALIKELVDLLGLARLEVPGYEADDVLASLAKKAEKEGYEVRILTADKDLYQLLSDRIHVLHPEGYLITPAWLWEKYGLRPDQWADYRALTGDESDNLPGVKGIGEKTARKLLEEWGSLEALLKNLDRLKPAIREKILAHMDDLKLSWDLAKVRTDLPLEVDFAKRREPDRERLRAFLERLEFGSLLHEFGLLESPKALEEAPWPPPEGAFVGFVLSRKEPMWADLLALAAARGGRVHRAPEPYKALRDLKEARGLLAKDLSVLALREGLGLPPGDDPMLLAYLLDPSNTTPEGVARRYGGEWTEEAGERAALSERLFANLWGRLEGEERLLWLYREVERPLSAVLAHMEATGVRLDVAYLRALSLEVAEEIARLEAEVFRLAGHPFNLNSRDQLERVLFDELGLPSIGKTEKTGKRSTSAAVLEALREAHPIVEKILQYRELTKLKSTYIDPLPDLIHPRTGRLHTRFNQTATATGRLSSSDPNLQNIPVRTPLGQRIRRAFIAEEGWLLVALDYSQIELRVLAHLSGDENLIRVFQEGRDIHTETASWMFGVPREAVDPLMRRAAKTINFGVLYGMSAHRLSQELAIPYEEAQAFIERYFQSFPKVRAWIEKTLEEGRRRGYVETLFGRRRYVPDLEARVKSVREAAERMAFNMPVQGTAADLMKLAMVKLFPRLEEMGARMLLQVHDELVLEAPKERAEAVARLAKEVMEGVYPLAVPLEVEVGIGEDWLSAKE

SEQ ID NO: 20 - protein, 832 aa, synthetic construct
  REGION 1..832: note = Synthetic: S543V
MRGMLPLFEPKGRVLLVDGHHLAYRTFHALKGLTTSRGEPVQAVYGFAKSLLKALKEDGDAVIVVFDAKAPSFRHEAYGGYKAGRAPTPEDFPRQLALIKELVDLLGLARLEVPGYEADDVLASLAKKAEKEGYEVRILTADKDLYQLLSDRIHVLHPEGYLITPAWLWEKYGLRPDQWADYRALTGDESDNLPGVKGIGEKTARKLLEEWGSLEALLKNLDRLKPAIREKILAHMDDLKLSWDLAKVRTDLPLEVDFAKRREPDRERLRAFLERLEFGSLLHEFGLLESPKALEEAPWPPPEGAFVGFVLSRKEPMWADLLALAAARGGRVHRAPEPYKALRDLKEARGLLAKDLSVLALREGLGLPPGDDPMLLAYLLDPSNTTPEGVARRYGGEWTEEAGERAALSERLFANLWGRLEGEERLLWLYREVERPLSAVLAHMEATGVRLDVAYLRALSLEVAEEIARLEAEVFRLAGHPFNLNSRDQLERVLFDELGLPAIGKTEKTGKRSTSAAVLEALREAHPIVEKILQYRELTKLKVTYIDPLPDLIHPRTGRLHTRFNQTATATGRLSSSDPNLQNIPVRTPLGQRIRRAFIAEEGWLLVALDYSQIELRVLAHLSGDENLIRVFQEGRDIHTETASWMFGVPREAVDPLMRRAAKTINFGVLYGMSAHRLSQELAIPYEEAQAFIERYFQSFPKVRAWIEKTLEEGRRRGYVETLFGRRRYVPDLEARVKSVREAAERMAFNMPVQGTAADLMKLAMVKLFPRLEEMGARMLLQVHDELVLEAPKERAEAVARLAKEVMEGVYPLAVPLEVEVGIGEDWLSAKE

SEQ ID NO: 21 - protein, 832 aa, synthetic construct
  REGION 1..832: note = Synthetic: D578E
MRGMLPLFEPKGRVLLVDGHHLAYRTFHALKGLTTSRGEPVQAVYGFAKSLLKALKEDGDAVIVVFDAKAPSFRHEAYGGYKAGRAPTPEDFPRQLALIKELVDLLGLARLEVPGYEADDVLASLAKKAEKEGYEVRILTADKDLYQLLSDRIHVLHPEGYLITPAWLWEKYGLRPDQWADYRALTGDESDNLPGVKGIGEKTARKLLEEWGSLEALLKNLDRLKPAIREKILAHMDDLKLSWDLAKVRTDLPLEVDFAKRREPDRERLRAFLERLEFGSLLHEFGLLESPKALEEAPWPPPEGAFVGFVLSRKEPMWADLLALAAARGGRVHRAPEPYKALRDLKEARGLLAKDLSVLALREGLGLPPGDDPMLLAYLLDPSNTTPEGVARRYGGEWTEEAGERAALSERLFANLWGRLEGEERLLWLYREVERPLSAVLAHMEATGVRLDVAYLRALSLEVAEEIARLEAEVFRLAGHPFNLNSRDQLERVLFDELGLPAIGKTEKTGKRSTSAAVLEALREAHPIVEKILQYRELTKLKSTYIDPLPDLIHPRTGRLHTRFNQTATATGRLSSSEPNLQNIPVRTPLGQRIRRAFIAEEGWLLVALDYSQIELRVLAHLSGDENLIRVFQEGRDIHTETASWMFGVPREAVDPLMRRAAKTINFGVLYGMSAHRLSQELAIPYEEAQAFIERYFQSFPKVRAWIEKTLEEGRRRGYVETLFGRRRYVPDLEARVKSVREAAERMAFNMPVQGTAADLMKLAMVKLFPRLEEMGARMLLQVHDELVLEAPKERAEAVARLAKEVMEGVYPLAVPLEVEVGIGEDWLSAKE

SEQ ID NO: 22 - protein, 832 aa, synthetic construct
  REGION 1..832: note = Synthetic: R593G
MRGMLPLFEPKGRVLLVDGHHLAYRTFHALKGLTTSRGEPVQAVYGFAKSLLKALKEDGDAVIVVFDAKAPSFRHEAYGGYKAGRAPTPEDFPRQLALIKELVDLLGLARLEVPGYEADDVLASLAKKAEKEGYEVRILTADKDLYQLLSDRIHVLHPEGYLITPAWLWEKYGLRPDQWADYRALTGDESDNLPGVKGIGEKTARKLLEEWGSLEALLKNLDRLKPAIREKILAHMDDLKLSWDLAKVRTDLPLEVDFAKRREPDRERLRAFLERLEFGSLLHEFGLLESPKALEEAPWPPPEGAFVGFVLSRKEPMWADLLALAAARGGRVHRAPEPYKALRDLKEARGLLAKDLSVLALREGLGLPPGDDPMLLAYLLDPSNTTPEGVARRYGGEWTEEAGERAALSERLFANLWGRLEGEERLLWLYREVERPLSAVLAHMEATGVRLDVAYLRALSLEVAEEIARLEAEVFRLAGHPFNLNSRDQLERVLFDELGLPAIGKTEKTGKRSTSAAVLEALREAHPIVEKILQYRELTKLKSTYIDPLPDLIHPRTGRLHTRFNQTATATGRLSSSDPNLQNIPVRTPLGQGIRRAFIAEEGWLLVALDYSQIELRVLAHLSGDENLIRVFQEGRDIHTETASWMFGVPREAVDPLMRRAAKTINFGVLYGMSAHRLSQELAIPYEEAQAFIERYFQSFPKVRAWIEKTLEEGRRRGYVETLFGRRRYVPDLEARVKSVREAAERMAFNMPVQGTAADLMKLAMVKLFPRLEEMGARMLLQVHDELVLEAPKERAEAVARLAKEVMEGVYPLAVPLEVEVGIGEDWLSAKE

SEQ ID NO: 23 - protein, 832 aa, synthetic construct
  REGION 1..832: note = Synthetic: L678F
MRGMLPLFEPKGRVLLVDGHHLAYRTFHALKGLTTSRGEPVQAVYGFAKSLLKALKEDGDAVIVVFDAKAPSFRHEAYGGYKAGRAPTPEDFPRQLALIKELVDLLGLARLEVPGYEADDVLASLAKKAEKEGYEVRILTADKDLYQLLSDRIHVLHPEGYLITPAWLWEKYGLRPDQWADYRALTGDESDNLPGVKGIGEKTARKLLEEWGSLEALLKNLDRLKPAIREKILAHMDDLKLSWDLAKVRTDLPLEVDFAKRREPDRERLRAFLERLEFGSLLHEFGLLESPKALEEAPWPPPEGAFVGFVLSRKEPMWADLLALAAARGGRVHRAPEPYKALRDLKEARGLLAKDLSVLALREGLGLPPGDDPMLLAYLLDPSNTTPEGVARRYGGEWTEEAGERAALSERLFANLWGRLEGEERLLWLYREVERPLSAVLAHMEATGVRLDVAYLRALSLEVAEEIARLEAEVFRLAGHPFNLNSRDQLERVLFDELGLPAIGKTEKTGKRSTSAAVLEALREAHPIVEKILQYRELTKLKSTYIDPLPDLIHPRTGRLHTRFNQTATATGRLSSSDPNLQNIPVRTPLGQRIRRAFIAEEGWLLVALDYSQIELRVLAHLSGDENLIRVFQEGRDIHTETASWMFGVPREAVDPLMRRAAKTINFGVLYGMSAHRFSQELAIPYEEAQAFIERYFQSFPKVRAWIEKTLEEGRRRGYVETLFGRRRYVPDLEARVKSVREAAERMAFNMPVQGTAADLMKLAMVKLFPRLEEMGARMLLQVHDELVLEAPKERAEAVARLAKEVMEGVYPLAVPLEVEVGIGEDWLSAKE

SEQ ID NO: 24 - protein, 832 aa, synthetic construct
  REGION 1..832: note = Synthetic: L678T
MRGMLPLFEPKGRVLLVDGHHLAYRTFHALKGLTTSRGEPVQAVYGFAKSLLKALKEDGDAVIVVFDAKAPSFRHEAYGGYKAGRAPTPEDFPRQLALIKELVDLLGLARLEVPGYEADDVLASLAKKAEKEGYEVRILTADKDLYQLLSDRIHVLHPEGYLITPAWLWEKYGLRPDQWADYRALTGDESDNLPGVKGIGEKTARKLLEEWGSLEALLKNLDRLKPAIREKILAHMDDLKLSWDLAKVRTDLPLEVDFAKRREPDRERLRAFLERLEFGSLLHEFGLLESPKALEEAPWPPPEGAFVGFVLSRKEPMWADLLALAAARGGRVHRAPEPYKALRDLKEARGLLAKDLSVLALREGLGLPPGDDPMLLAYLLDPSNTTPEGVARRYGGEWTEEAGERAALSERLFANLWGRLEGEERLLWLYREVERPLSAVLAHMEATGVRLDVAYLRALSLEVAEEIARLEAEVFRLAGHPFNLNSRDQLERVLFDELGLPAIGKTEKTGKRSTSAAVLEALREAHPIVEKILQYRELTKLKSTYIDPLPDLIHPRTGRLHTRFNQTATATGRLSSSDPNLQNIPVRTPLGQRIRRAFIAEEGWLLVALDYSQIELRVLAHLSGDENLIRVFQEGRDIHTETASWMFGVPREAVDPLMRRAAKTINFGVLYGMSAHRTSQELAIPYEEAQAFIERYFQSFPKVRAWIEKTLEEGRRRGYVETLFGRRRYVPDLEARVKSVREAAERMAFNMPVQGTAADLMKLAMVKLFPRLEEMGARMLLQVHDELVLEAPKERAEAVARLAKEVMEGVYPLAVPLEVEVGIGEDWLSAKE

SEQ ID NO: 25 - protein, 832 aa, synthetic construct
  REGION 1..832: note = Synthetic: S699W
MRGMLPLFEPKGRVLLVDGHHLAYRTFHALKGLTTSRGEPVQAVYGFAKSLLKALKEDGDAVIVVFDAKAPSFRHEAYGGYKAGRAPTPEDFPRQLALIKELVDLLGLARLEVPGYEADDVLASLAKKAEKEGYEVRILTADKDLYQLLSDRIHVLHPEGYLITPAWLWEKYGLRPDQWADYRALTGDESDNLPGVKGIGEKTARKLLEEWGSLEALLKNLDRLKPAIREKILAHMDDLKLSWDLAKVRTDLPLEVDFAKRREPDRERLRAFLERLEFGSLLHEFGLLESPKALEEAPWPPPEGAFVGFVLSRKEPMWADLLALAAARGGRVHRAPEPYKALRDLKEARGLLAKDLSVLALREGLGLPPGDDPMLLAYLLDPSNTTPEGVARRYGGEWTEEAGERAALSERLFANLWGRLEGEERLLWLYREVERPLSAVLAHMEATGVRLDVAYLRALSLEVAEEIARLEAEVFRLAGHPFNLNSRDQLERVLFDELGLPAIGKTEKTGKRSTSAAVLEALREAHPIVEKILQYRELTKLKSTYIDPLPDLIHPRTGRLHTRFNQTATATGRLSSSDPNLQNIPVRTPLGQRIRRAFIAEEGWLLVALDYSQIELRVLAHLSGDENLIRVFQEGRDIHTETASWMFGVPREAVDPLMRRAAKTINFGVLYGMSAHRLSQELAIPYEEAQAFIERYFQWFPKVRAWIEKTLEEGRRRGYVETLFGRRRYVPDLEARVKSVREAAERMAFNMPVQGTAADLMKLAMVKLFPRLEEMGARMLLQVHDELVLEAPKERAEAVARLAKEVMEGVYPLAVPLEVEVGIGEDWLSAKE

SEQ ID NO: 26 - protein, 832 aa, synthetic construct
  REGION 1..832: note = Synthetic: E713W
MRGMLPLFEPKGRVLLVDGHHLAYRTFHALKGLTTSRGEPVQAVYGFAKSLLKALKEDGDAVIVVFDAKAPSFRHEAYGGYKAGRAPTPEDFPRQLALIKELVDLLGLARLEVPGYEADDVLASLAKKAEKEGYEVRILTADKDLYQLLSDRIHVLHPEGYLITPAWLWEKYGLRPDQWADYRALTGDESDNLPGVKGIGEKTARKLLEEWGSLEALLKNLDRLKPAIREKILAHMDDLKLSWDLAKVRTDLPLEVDFAKRREPDRERLRAFLERLEFGSLLHEFGLLESPKALEEAPWPPPEGAFVGFVLSRKEPMWADLLALAAARGGRVHRAPEPYKALRDLKEARGLLAKDLSVLALREGLGLPPGDDPMLLAYLLDPSNTTPEGVARRYGGEWTEEAGERAALSERLFANLWGRLEGEERLLWLYREVERPLSAVLAHMEATGVRLDVAYLRALSLEVAEEIARLEAEVFRLAGHPFNLNSRDQLERVLFDELGLPAIGKTEKTGKRSTSAAVLEALREAHPIVEKILQYRELTKLKSTYIDPLPDLIHPRTGRLHTRFNQTATATGRLSSSDPNLQNIPVRTPLGQRIRRAFIAEEGWLLVALDYSQIELRVLAHLSGDENLIRVFQEGRDIHTETASWMFGVPREAVDPLMRRAAKTINFGVLYGMSAHRLSQELAIPYEEAQAFIERYFQSFPKVRAWIEKTLEWGRRRGYVETLFGRRRYVPDLEARVKSVREAAERMAFNMPVQGTAADLMKLAMVKLFPRLEEMGARMLLQVHDELVLEAPKERAEAVARLAKEVMEGVYPLAVPLEVEVGIGEDWLSAKE

SEQ ID NO: 27 - protein, 832 aa, synthetic construct
  REGION 1..832: note = Synthetic: V737A
MRGMLPLFEPKGRVLLVDGHHLAYRTFHALKGLTTSRGEPVQAVYGFAKSLLKALKEDGDAVIVVFDAKAPSFRHEAYGGYKAGRAPTPEDFPRQLALIKELVDLLGLARLEVPGYEADDVLASLAKKAEKEGYEVRILTADKDLYQLLSDRIHVLHPEGYLITPAWLWEKYGLRPDQWADYRALTGDESDNLPGVKGIGEKTARKLLEEWGSLEALLKNLDRLKPAIREKILAHMDDLKLSWDLAKVRTDLPLEVDFAKRREPDRERLRAFLERLEFGSLLHEFGLLESPKALEEAPWPPPEGAFVGFVLSRKEPMWADLLALAAARGGRVHRAPEPYKALRDLKEARGLLAKDLSVLALREGLGLPPGDDPMLLAYLLDPSNTTPEGVARRYGGEWTEEAGERAALSERLFANLWGRLEGEERLLWLYREVERPLSAVLAHMEATGVRLDVAYLRALSLEVAEEIARLEAEVFRLAGHPFNLNSRDQLERVLFDELGLPAIGKTEKTGKRSTSAAVLEALREAHPIVEKILQYRELTKLKSTYIDPLPDLIHPRTGRLHTRFNQTATATGRLSSSDPNLQNIPVRTPLGQRIRRAFIAEEGWLLVALDYSQIELRVLAHLSGDENLIRVFQEGRDIHTETASWMFGVPREAVDPLMRRAAKTINFGVLYGMSAHRLSQELAIPYEEAQAFIERYFQSFPKVRAWIEKTLEEGRRRGYVETLFGRRRYVPDLEARAKSVREAAERMAFNMPVQGTAADLMKLAMVKLFPRLEEMGARMLLQVHDELVLEAPKERAEAVARLAKEVMEGVYPLAVPLEVEVGIGEDWLSAKE

SEQ ID NO: 28 - protein, 832 aa, synthetic construct
  REGION 1..832: note = Synthetic: E745T
MRGMLPLFEPKGRVLLVDGHHLAYRTFHALKGLTTSRGEPVQAVYGFAKSLLKALKEDGDAVIVVFDAKAPSFRHEAYGGYKAGRAPTPEDFPRQLALIKELVDLLGLARLEVPGYEADDVLASLAKKAEKEGYEVRILTADKDLYQLLSDRIHVLHPEGYLITPAWLWEKYGLRPDQWADYRALTGDESDNLPGVKGIGEKTARKLLEEWGSLEALLKNLDRLKPAIREKILAHMDDLKLSWDLAKVRTDLPLEVDFAKRREPDRERLRAFLERLEFGSLLHEFGLLESPKALEEAPWPPPEGAFVGFVLSRKEPMWADLLALAAARGGRVHRAPEPYKALRDLKEARGLLAKDLSVLALREGLGLPPGDDPMLLAYLLDPSNTTPEGVARRYGGEWTEEAGERAALSERLFANLWGRLEGEERLLWLYREVERPLSAVLAHMEATGVRLDVAYLRALSLEVAEEIARLEAEVFRLAGHPFNLNSRDQLERVLFDELGLPAIGKTEKTGKRSTSAAVLEALREAHPIVEKILQYRELTKLKSTYIDPLPDLIHPRTGRLHTRFNQTATATGRLSSSDPNLQNIPVRTPLGQRIRRAFIAEEGWLLVALDYSQIELRVLAHLSGDENLIRVFQEGRDIHTETASWMFGVPREAVDPLMRRAAKTINFGVLYGMSAHRLSQELAIPYEEAQAFIERYFQSFPKVRAWIEKTLEEGRRRGYVETLFGRRRYVPDLEARVKSVREAATRMAFNMPVQGTAADLMKLAMVKLFPRLEEMGARMLLQVHDELVLEAPKERAEAVARLAKEVMEGVYPLAVPLEVEVGIGEDWLSAKE

SEQ ID NO: 29 - protein, 832 aa, synthetic construct
  REGION 1..832: note = Synthetic: L763F
MRGMLPLFEPKGRVLLVDGHHLAYRTFHALKGLTTSRGEPVQAVYGFAKSLLKALKEDGDAVIVVFDAKAPSFRHEAYGGYKAGRAPTPEDFPRQLALIKELVDLLGLARLEVPGYEADDVLASLAKKAEKEGYEVRILTADKDLYQLLSDRIHVLHPEGYLITPAWLWEKYGLRPDQWADYRALTGDESDNLPGVKGIGEKTARKLLEEWGSLEALLKNLDRLKPAIREKILAHMDDLKLSWDLAKVRTDLPLEVDFAKRREPDRERLRAFLERLEFGSLLHEFGLLESPKALEEAPWPPPEGAFVGFVLSRKEPMWADLLALAAARGGRVHRAPEPYKALRDLKEARGLLAKDLSVLALREGLGLPPGDDPMLLAYLLDPSNTTPEGVARRYGGEWTEEAGERAALSERLFANLWGRLEGEERLLWLYREVERPLSAVLAHMEATGVRLDVAYLRALSLEVAEEIARLEAEVFRLAGHPFNLNSRDQLERVLFDELGLPAIGKTEKTGKRSTSAAVLEALREAHPIVEKILQYRELTKLKSTYIDPLPDLIHPRTGRLHTRFNQTATATGRLSSSDPNLQNIPVRTPLGQRIRRAFIAEEGWLLVALDYSQIELRVLAHLSGDENLIRVFQEGRDIHTETASWMFGVPREAVDPLMRRAAKTINFGVLYGMSAHRLSQELAIPYEEAQAFIERYFQSFPKVRAWIEKTLEEGRRRGYVETLFGRRRYVPDLEARVKSVREAAERMAFNMPVQGTAADLMKFAMVKLFPRLEEMGARMLLQVHDELVLEAPKERAEAVARLAKEVMEGVYPLAVPLEVEVGIGEDWLSAKE

SEQ ID NO: 30 - protein, 832 aa, synthetic construct
  REGION 1..832: note = Synthetic: E790G
MRGMLPLFEPKGRVLLVDGHHLAYRTFHALKGLTTSRGEPVQAVYGFAKSLLKALKEDGDAVIVVFDAKAPSFRHEAYGGYKAGRAPTPEDFPRQLALIKELVDLLGLARLEVPGYEADDVLASLAKKAEKEGYEVRILTADKDLYQLLSDRIHVLHPEGYLITPAWLWEKYGLRPDQWADYRALTGDESDNLPGVKGIGEKTARKLLEEWGSLEALLKNLDRLKPAIREKILAHMDDLKLSWDLAKVRTDLPLEVDFAKRREPDRERLRAFLERLEFGSLLHEFGLLESPKALEEAPWPPPEGAFVGFVLSRKEPMWADLLALAAARGGRVHRAPEPYKALRDLKEARGLLAKDLSVLALREGLGLPPGDDPMLLAYLLDPSNTTPEGVARRYGGEWTEEAGERAALSERLFANLWGRLEGEERLLWLYREVERPLSAVLAHMEATGVRLDVAYLRALSLEVAEEIARLEAEVFRLAGHPFNLNSRDQLERVLFDELGLPAIGKTEKTGKRSTSAAVLEALREAHPIVEKILQYRELTKLKSTYIDPLPDLIHPRTGRLHTRFNQTATATGRLSSSDPNLQNIPVRTPLGQRIRRAFIAEEGWLLVALDYSQIELRVLAHLSGDENLIRVFQEGRDIHTETASWMFGVPREAVDPLMRRAAKTINFGVLYGMSAHRLSQELAIPYEEAQAFIERYFQSFPKVRAWIEKTLEEGRRRGYVETLFGRRRYVPDLEARVKSVREAAERMAFNMPVQGTAADLMKLAMVKLFPRLEEMGARMLLQVHDELVLGAPKERAEAVARLAKEVMEGVYPLAVPLEVEVGIGEDWLSAKE

SEQ ID NO: 31 - protein, 832 aa, synthetic construct
  REGION 1..832: note = Synthetic: E794C
MRGMLPLFEPKGRVLLVDGHHLAYRTFHALKGLTTSRGEPVQAVYGFAKSLLKALKEDGDAVIVVFDAKAPSFRHEAYGGYKAGRAPTPEDFPRQLALIKELVDLLGLARLEVPGYEADDVLASLAKKAEKEGYEVRILTADKDLYQLLSDRIHVLHPEGYLITPAWLWEKYGLRPDQWADYRALTGDESDNLPGVKGIGEKTARKLLEEWGSLEALLKNLDRLKPAIREKILAHMDDLKLSWDLAKVRTDLPLEVDFAKRREPDRERLRAFLERLEFGSLLHEFGLLESPKALEEAPWPPPEGAFVGFVLSRKEPMWADLLALAAARGGRVHRAPEPYKALRDLKEARGLLAKDLSVLALREGLGLPPGDDPMLLAYLLDPSNTTPEGVARRYGGEWTEEAGERAALSERLFANLWGRLEGEERLLWLYREVERPLSAVLAHMEATGVRLDVAYLRALSLEVAEEIARLEAEVFRLAGHPFNLNSRDQLERVLFDELGLPAIGKTEKTGKRSTSAAVLEALREAHPIVEKILQYRELTKLKSTYIDPLPDLIHPRTGRLHTRFNQTATATGRLSSSDPNLQNIPVRTPLGQRIRRAFIAEEGWLLVALDYSQIELRVLAHLSGDENLIRVFQEGRDIHTETASWMFGVPREAVDPLMRRAAKTINFGVLYGMSAHRLSQELAIPYEEAQAFIERYFQSFPKVRAWIEKTLEEGRRRGYVETLFGRRRYVPDLEARVKSVREAAERMAFNMPVQGTAADLMKLAMVKLFPRLEEMGARMLLQVHDELVLEAPKCRAEAVARLAKEVMEGVYPLAVPLEVEVGIGEDWLSAKE

SEQ ID NO: 32 - protein, 832 aa, synthetic construct
  REGION 1..832: note = Synthetic: E805I
MRGMLPLFEPKGRVLLVDGHHLAYRTFHALKGLTTSRGEPVQAVYGFAKSLLKALKEDGDAVIVVFDAKAPSFRHEAYGGYKAGRAPTPEDFPRQLALIKELVDLLGLARLEVPGYEADDVLASLAKKAEKEGYEVRILTADKDLYQLLSDRIHVLHPEGYLITPAWLWEKYGLRPDQWADYRALTGDESDNLPGVKGIGEKTARKLLEEWGSLEALLKNLDRLKPAIREKILAHMDDLKLSWDLAKVRTDLPLEVDFAKRREPDRERLRAFLERLEFGSLLHEFGLLESPKALEEAPWPPPEGAFVGFVLSRKEPMWADLLALAAARGGRVHRAPEPYKALRDLKEARGLLAKDLSVLALREGLGLPPGDDPMLLAYLLDPSNTTPEGVARRYGGEWTEEAGERAALSERLFANLWGRLEGEERLLWLYREVERPLSAVLAHMEATGVRLDVAYLRALSLEVAEEIARLEAEVFRLAGHPFNLNSRDQLERVLFDELGLPAIGKTEKTGKRSTSAAVLEALREAHPIVEKILQYRELTKLKSTYIDPLPDLIHPRTGRLHTRFNQTATATGRLSSSDPNLQNIPVRTPLGQRIRRAFIAEEGWLLVALDYSQIELRVLAHLSGDENLIRVFQEGRDIHTETASWMFGVPREAVDPLMRRAAKTINFGVLYGMSAHRLSQELAIPYEEAQAFIERYFQSFPKVRAWIEKTLEEGRRRGYVETLFGRRRYVPDLEARVKSVREAAERMAFNMPVQGTAADLMKLAMVKLFPRLEEMGARMLLQVHDELVLEAPKERAEAVARLAKIVMEGVYPLAVPLEVEVGIGEDWLSAKE

SEQ ID NO: 33 - protein, 832 aa, synthetic construct
  REGION 1..832: note = Synthetic: L828A
MRGMLPLFEPKGRVLLVDGHHLAYRTFHALKGLTTSRGEPVQAVYGFAKSLLKALKEDGDAVIVVFDAKAPSFRHEAYGGYKAGRAPTPEDFPRQLALIKELVDLLGLARLEVPGYEADDVLASLAKKAEKEGYEVRILTADKDLYQLLSDRIHVLHPEGYLITPAWLWEKYGLRPDQWADYRALTGDESDNLPGVKGIGEKTARKLLEEWGSLEALLKNLDRLKPAIREKILAHMDDLKLSWDLAKVRTDLPLEVDFAKRREPDRERLRAFLERLEFGSLLHEFGLLESPKALEEAPWPPPEGAFVGFVLSRKEPMWADLLALAAARGGRVHRAPEPYKALRDLKEARGLLAKDLSVLALREGLGLPPGDDPMLLAYLLDPSNTTPEGVARRYGGEWTEEAGERAALSERLFANLWGRLEGEERLLWLYREVERPLSAVLAHMEATGVRLDVAYLRALSLEVAEEIARLEAEVFRLAGHPFNLNSRDQLERVLFDELGLPAIGKTEKTGKRSTSAAVLEALREAHPIVEKILQYRELTKLKSTYIDPLPDLIHPRTGRLHTRFNQTATATGRLSSSDPNLQNIPVRTPLGQRIRRAFIAEEGWLLVALDYSQIELRVLAHLSGDENLIRVFQEGRDIHTETASWMFGVPREAVDPLMRRAAKTINFGVLYGMSAHRLSQELAIPYEEAQAFIERYFQSFPKVRAWIEKTLEEGRRRGYVETLFGRRRYVPDLEARVKSVREAAERMAFNMPVQGTAADLMKLAMVKLFPRLEEMGARMLLQVHDELVLEAPKERAEAVARLAKEVMEGVYPLAVPLEVEVGIGEDWASAKE

SEQ ID NO: 34 - protein, 832 aa, synthetic construct
  REGION 1..832: note = Synthetic: (REF POLY) - (Taq-LR1) D732R
MRGMLPLFEPKGRVLLVDGHHLAYRTFHALKGLTTSRGEPVQAVYGFAKSLLKALKEDGDAVIVVFDAKAPSFRHEAYGGYKAGRAPTPEDFPRQLALIKELVDLLGLARLEVPGYEADDVLASLAKKAEKEGYEVRILTADKDLYQLLSDRIHVLHPEGYLITPAWLWEKYGLRPDQWADYRALTGDESDNLPGVKGIGEKTARKLLEEWGSLEALLKNLDRLKPAIREKILAHMDDLKLSWDLAKVRTDLPLEVDFAKRREPDRERLRAFLERLEFGSLLHEFGLLESPKALEEAPWPPPEGAFVGFVLSRKEPMWADLLALAAARGGRVHRAPEPYKALRDLKEARGLLAKDLSVLALREGLGLPPGDDPMLLAYLLDPSNTTPEGVARRYGGEWTEEAGERAALSERLFANLWGRLEGEERLLWLYREVERPLSAVLAHMEATGVRLDVAYLRALSLEVAEEIARLEAEVFRLAGHPFNLNSRDQLERVLFDELGLPAIGKTEKTGKRSTSAAVLEALREAHPIVEKILQYRELTKLKSTYIDPLPDLIHPRTGRLHTRFNQTATATGRLSSSDPNLQNIPVRTPLGQRIRRAFIAEEGWLLVALDYSQIELRVLAHLSGDENLIRVFQEGRDIHTETASWMFGVPREAVDPLMRRAAKTINFGVLYGMSAHRLSQELAIPYEEAQAFIERYFQSFPKVRAWIEKTLEEGRRRGYVETLFGRRRYVPRLEARVKSVREAAERMAFNMPVQGTAADLMKLAMVKLFPRLEEMGARMLLQVHDELVLEAPKERAEAVARLAKEVMEGVYPLAVPLEVEVGIGEDWLSAKE

SEQ ID NO: 35-36 - skipped (2 entries)

SEQ ID NO: 37 - protein, 4 aa, synthetic construct
  REGION 1..4: note = Synthetic peptide
VHDE

SEQ ID NO: 38 - protein, 8 aa, synthetic construct
  REGION 1..8: note = Synthetic peptide
  REGION 2..3: note = misc_feature - Xaa can be any naturally occurring amino acid
DXXSLYPS

SEQ ID NO: 39 - protein, 9 aa, synthetic construct
  REGION 1..9: note = Synthetic peptide
  REGION 2..4: note = misc_feature - Xaa can be any naturally occurring amino acid
  SITE 7: note = misc_feature - Xaa can be any naturally occurring amino acid
KXXXNSXYG

SEQ ID NO: 40 - protein, 6 aa, synthetic construct
  REGION 1..6: note = Synthetic peptide
YGDTDS

SEQ ID NO: 41-44 - skipped (4 entries)